European Patent Application EP 4 800 117 A1, published September 2, 2026. Title: METHOD FOR PRODUCING NMN AND METHOD FOR PRODUCING NAD. Applicant: Oriental Yeast Co., Ltd. Application JP. The sequence listing filed with the application follows.

SEQUENCE LISTING (28 sequences)

SEQ ID NO: 1 - protein, 463 aa, Sandaracinus amylolyticus
MITMEGSNLLLGTDSYKVTHWRQYPPGTTRVSSFLESRGGVYPSVVFFGLQYLLDRHFAGVVVTEDRIAEAREIFAAHFGDPTLFHEAGWRHVLDAHGGRLPVEIRAVPEGTVVPVSNVLMTIENTDPRVPWLTNYLESLLLQVWYPCTVATQSREMRRTITAHLEKTGTPSLVGFELHDFGLRGSTSHESAAIGGAAHLVSFEGTDTIPALLLARRHYGEPMAGFSIPAAEHSTITSWGRDRESSAYRNMLESYPRGLVAVVSDSYDVYRACEQLWGRELRELVLSRDGTLVVRPDSGHPPEVVCRVLEILGRAFGTAINAKGYRVLDPHVRVIQGDGIDPVMIAEILAAMSERGWSADNVAFGSGGALLQKVHRDTQNLAIKCSAVEIDGAWRPVMKDPVTDPGKRSKSGRLALVREAGAFRTVARGDSGHPGDLLEPVFRDGEILRRQTLSDIRRRALEG

SEQ ID NO: 2 - protein, 98 aa, Sandaracinus amylolyticus
NLLLGTDSYKVTHWRQYPPGTTRVSSFLESRGGVYPSVVFFGLQYLLDRHFAGVVVTEDRIAEAREIFAAHFGDPTLFHEAGWRHVLDAHGGRLPVEI

SEQ ID NO: 3 - protein, 244 aa, Sandaracinus amylolyticus
FELHDFGLRGSTSHESAAIGGAAHLVSFEGTDTIPALLLARRHYGEPMAGFSIPAAEHSTITSWGRDRESSAYRNMLESYPRGLVAVVSDSYDVYRACEQLWGRELRELVLSRDGTLVVRPDSGHPPEVVCRVLEILGRAFGTAINAKGYRVLDPHVRVIQGDGIDPVMIAEILAAMSERGWSADNVAFGSGGALLQKVHRDTQNLAIKCSAVEIDGAWRPVMKDPVTDPGKRSKSGRLALVRE

SEQ ID NO: 4 - protein, 462 aa, Convivina intestine
MTNIILATDAYKLTHHLQYPQNITKLYSYGEARQGGRYDHISWFGMSMILNDYFTQPVTDAMIDEAQKVAELTFGNDVYFNRPVWEKVRDLGHFPVKIKALPEGMVVPTGTALFTIESTQSWFATSLNALETILMHVWYPTTIATNSMYIKKRLAPLVEKSGSMDNLPLMVNDFGLRGATSLESGERGGSAHLLHFRGSDNMAASRYFASVYGLEGRALSIWATEHSVATAYGEGQGELDYLNAQLDRTPEEAPVSIVIDSYDTFNFVQNVVGSPAMKERIKNRLGRVVLRPDSGDPQTVDLQILDLLAEIFGTSLNEKGYRVLNHNVGLIQGDGMNADTMIELYQALLDHGWSSDNLVVGSGGGLLQEGFTRDTERFAIKEAYAENSAGEHLQIQKRPKTDPSKVSKSGRMKVIYDDQGQIITVPADHPGQDLLETVYDNGYMKQIDVNSMLARAENFHDF

SEQ ID NO: 5 - protein, 96 aa, Convivina intestine
NIILATDAYKLTHHLQYPQNITKLYSYGEARQGGRYDHISWFGMSMILNDYFTQPVTDAMIDEAQKVAELTFGNDVYFNRPVWEKVRDLGHFPVKI

SEQ ID NO: 6 - protein, 272 aa, Convivina intestine
VNDFGLRGATSLESGERGGSAHLLHFRGSDNMAASRYFASVYGLEGRALSIWATEHSVATAYGEGQGELDYLNAQLDRTPEEAPVSIVIDSYDTFNFVQNVVGSPAMKERIKNRLGRVVLRPDSGDPQTVDLQILDLLAEIFGTSLNEKGYRVLNHNVGLIQGDGMNADTMIELYQALLDHGWSSDNLVVGSGGGLLQEGFTRDTERFAIKEAYAENSAGEHLQIQKRPKTDPSKVSKSGRMKVIYDDQGQIITVPADHPGQDLLETVYDNG

SEQ ID NO: 7 - protein, 410 aa, Escherichia coli
MSSFDYLKTAIKQQGCTLQQVADASGMTKGYLSQLLNAKIKSPSAQKLEALHRFLGLEFPRQKKTIGVVFGKFYPLHTGHIYLIQRACSQVDELHIIMGFDDTRDRALFEDSAMSQQPTVPDRLRWLLQTFKYQKNIRIHAFNEEGMEPYPHGWDVWSNGIKKFMAEKGIQPDLIYTSEEADAPQYMEHLGIETVLVDPKRTFMSISGAQIRENPFRYWEYIPTEVKPFFVRTVAILGGESSGKSTLVNKLANIFNTTSAWEYGRDYVFSHLGGDEIALQYSDYDKIALGHAQYIDFAVKYANKVAFIDTDFVTTQAFCKKYEGREHPFVQALIDEYRFDLVILLENNTPWVADGLRSLGSSVDRKEFQNLLVEMLEENNIEFVRVEEEDYDSRFLRCVELVREMMGEQR

SEQ ID NO: 8 - protein, 285 aa, synthetic construct
LSGAFAGFLSGVAVCPLDVAKTRLQAQGLQTRFENPYYRGIMGTLSTIVRDEGPRGLYKGLVPIVLGYFPTWMIYFSVYEFSKKFFHGIFPQFDFVAQSCAAITAGAASTTLTNPIWVVKTRLMLQSNLGEHPTHYKGTFDAFRKLFYQEGFKALYAGLVPSLLGLFHVAIHFPIYEDLKVRFHCYSRENNTNSINLQRLIMASSVSKMIASAVTYPHEILRTRMQLKSDIPDSIQRRLFPLIKATYAQEGLKGFYSGFTTNLVRTIPASAITLVSFEYFRNRLE

SEQ ID NO: 9 - protein, 201 aa, Chlamydia trachomatis
VFFTATFLATLVLTPLFGWLVSCWPRRVIMPLIYLFFIALQMVFILLFLNKNLLSPKVLGIFFYVWVSIFNLFVVSVFWSFMTDIWSDPQARRLFPIIGLGGTLGAVMGPIITRSLVEFIGLALLLAVSAAFLAIAVICIMLLGKWAHDHGAHRNELGSESAIGGGMLDGLKQIFSNPFIASMSLMMLLNDAIGTIAYVLI

SEQ ID NO: 10 - protein, 380 aa, Escherichia coli
PLCLVLYEFSTYIGNDMIQPGMLAVVEQYQAGIDWVPTSMTAYLAGGMFLQWLLGPLSDRIGRRPVMLAGVVWFIVTCLAILLAQNIEQFTLLRFLQGISLCFIGAVGYAAIQESFEEAVCIKITALMANVALIAPLLGPLVGAAWIHVLPWEGMFVLFAALAAISFFGLQRAMPETATRIGEKLSLKELGRDYKLVLKNGRFVAGALALGFVSLPLLAWIAQSPIIIITGEQLSSYEYGLLQVPIFGALIAGNLLLARLTSRRTVRSLIIMGGWPIMIGLLVAAAATVISSHAYLWMTAGLSIYAFGIGLANAGLVRLTLFASDMSKGTVSAAMGMLQMLIFTVGIEISKHAWLNGGNGLFNLFNLVNGILWLSLMVIF

SEQ ID NO: 11 - protein, 436 aa, Escherichia coli
AAMAFFMQALDATILNTALPAIAHSLNRSPLAMQSAIISYTLTVAMLIPVSGWLADRFGTRRIFTLAVSLFTLGSLACALSNSLPQLVVFRVIQGIGGAMMMPVARLALLRAYPRNELLPVLNFVAMPGLVGPILGPVLGGVLVTWATWHWIFLINIPIGIAGLLYARKHMPNFTTARRRFDITGFLLFGLSLVLFSSGIELFGEKIVASWIALTVIVTSIGLLLLYILHARRTPNPLISLDLFKTRTFSIGIVGNIATRLGTGCVPFLMPLMLQVGFGYQAFIAGCMMAPTALGSIIAKSMVTQVLRRLGYRHTLVGITVIIGLMIAQFSLQSPAMAIWMLILPLFILGMAMSTQFTAMNTITLADLTDDNASSGNSVLAVTQQLSISLGVAVSAAVLRVYEGMEGTTTVEQFHYTFITMGIITVASAAMFMLLK

SEQ ID NO: 12 - protein, 397 aa, Corynebacterium stationis
LMLTMLMSSLGQMIFGSALPTIVGELGGVDQMSWVISAFMVTMTIAMPLAGQLGDRMGRKWVYISGISIFVIGSTLGGFANGMGMLITGRAIQGFGAGIMMISSQSIVAEVVSARERGKFMGIMGGVFGVSSVLGPVLGGWFTDGPGWRWGLWINIPLGLLAIIVCAFVLKLRVGEQGFKGFDWMGFAAIAITTSTLILLTTWGGSEYEWTSPTILSMAAVVIVGALLTVFIESRASQPLIPVQLFKNRNMVLTTLAGTVLGLAMMGVLGYMPTYLQMVHTLTPTEAGLMMIPMMVGMIGVSTGVGFIIAKTGNYKYYPIAGLAITAFALWWMSQMTVETSLTGIGVRFLVFGVGLGFVMQVLVLIVQNSFPVSQVGTATAANNFFRQIGSALGASI

SEQ ID NO: 13 - protein, 287 aa, Corynebacterium stationis
SALGNSIAGIVRPWIVLERTDDPAAGLVAAAVAVPSVIFASLGGYLIDTVGRKPISVTSDIISGASVAGVVLVDQTLGLTIAWFIALGIIGGVRDIPGMAARPALVGDVSQASGKTVDYIAGLNQAILGVAFLVGPAVAAVLLAALNSSLVRIITAACSFLAALLTTFLRLAKRELTEKEKQAAAADNALNLQALKSWDRLSVPHPFGCLAFSFYAIGMMISGAGIAKVGTSRRRLVWAVAIGVEAIGFAMMAALGVSWLVVIGCGISGLAGGRLSPLQMVLIILSI

SEQ ID NO: 14 - protein, 397 aa, synthetic construct
LMLTMLMSSLEQMIFGSALPTIVGELGGVDQMSWVISAFMVTMTIAMPLAGQLGDRMGRKWVYISGISIFVIGSTLGGFANGMGMLITGRAIQGFGAGIMMISSQSIVAEVVSARERGKFMGIMGGVFGVSSVLGPVLGGWFTDGPGWRWGLWINIPLGLLAIIVCAFVLKLRVGEQGFKGFDWMGFAAIAITTSTLILLTTWGGSEYEWTSPTILSMAAVVIVGALLTVFIESRASQPLIPVQLFKNRNMVLTTLAGTVLGLAMMGVLGYMPTYLQMVHTLTPTEAGLMMIPMMVGMIGVSTGVGFIIAKTGNYKYYPIAGLAITAFALWWMSQMTVETSLTGIGVRFLVFGVGLGFVMQVLVLIVQNSFPVSQVGTATAANNFFRQIGSALGASI

SEQ ID NO: 15 - protein, 522 aa, Corynebacterium tuberculostearicum
MVDTATKAPSQGQSRADNLGLIFSALMLTMLMSSLGQMIFSSALPTIVGELGGVDHMSWVISAFLVTMTIAMPISGKLGDMLGRKWLYIGGIATFVVGSTLGGFANSMTLLIIARAVQGFGAGFMMISSQSIIAEVTSSRERGKFMGIMGGVFGLSSVLGPVLGGWFTDGPGWRWGMWMNIPLGILAIIVCTLVLHLRVGDADMKRFDWLGATFIAITTASLILMTTWGGTEYEWGSSMILTLGAITIIGAIITVFVELRAKEPLIPVRLFKNRNMALTTLSGVVLGLAMFGVLGYMPTYLQMVHTLTPTKAGLMMIPMMVGLIGTSTGVGFIIARTGHYKVYPIIGLAITAGALFWMSHLSVETSLKQLGCEFLVFGIGLGMVIQVLVLIVQNSFPLSQVGTATAANNFFRQIGSALGASLVGSMFIHNMQDEMATRMPEAFQKMGPEGAAYAEKFGDANGGANSLTPDLVASFPKPIEEAILNSYNDGLTPVIALMVPLVIVALILLLPLREERLKETID

SEQ ID NO: 16 - protein, 522 aa, synthetic construct
MVDTATKAPSQGQSRADNLGLIFSALMLTMLMSSLEQMIFSSALPTIVGELGGVDHMSWVISAFLVTMTIAMPISGKLGDMLGRKWLYIGGIATFVVGSTLGGFANSMTLLIIARAVQGFGAGFMMISSQSIIAEVTSSRERGKFMGIMGGVFGLSSVLGPVLGGWFTDGPGWRWGMWMNIPLGILAIIVCTLVLHLRVGDADMKRFDWLGATFIAITTASLILMTTWGGTEYEWGSSMILTLGAITIIGAIITVFVELRAKEPLIPVRLFKNRNMALTTLSGVVLGLAMFGVLGYMPTYLQMVHTLTPTKAGLMMIPMMVGLIGTSTGVGFIIARTGHYKVYPIIGLAITAGALFWMSHLSVETSLKQLGCEFLVFGIGLGMVIQVLVLIVQNSFPLSQVGTATAANNFFRQIGSALGASLVGSMFIHNMQDEMATRMPEAFQKMGPEGAAYAEKFGDANGGANSLTPDLVASFPKPIEEAILNSYNDGLTPVIALMVPLVIVALILLLPLREERLKETID

SEQ ID NO: 17 - protein, 512 aa, Corynebacterium sp.
MVDTQHKGPNVGLVFTALLITMLMSSLGQMIFSSALPTIVGELGGVEHMSWVISAFMVTMTIALPLYGKLGDGLGRKWFYISGIAFFIIGSALGGFANTMTLLIIGRAVQGFGAGAMMINSQAIIAEVVPARERGKYMGVMGAVFGISSVLGPVLGGWFTDGPGWRWGLWMNIPLGLLAMTVASIVLDLSKGNRDGFRFDWLGATFMAVSTSTLILATTWGGLQYPWGSPRIVGLLVTSAVAAALFVVVELRATDPLVPMHLFRNRNMALTTAASVVLGISMTGVMAYLPTYLQMVHSMTPTEAGLMMIPMVGGMIITSIGIGALISRTGSYKIFPIVGLGVVALGCYLLSRLTVDTGLWTLGLYIFIYGFGLGMVMQVLILIVQNSFPIAVVGTATAANNFFRQIGMSVGASVVGTVFIHNMQQNMEERLPGALAALGPEGAKYAESFSDGATQSMTPSAVNQLPQPLHDAISTSYNDGLTPIFLLLIPLVVAAALLLVPVHEDTLKETIE

SEQ ID NO: 18 - protein, 512 aa, synthetic construct
MVDTQHKGPNVGLVFTALLITMLMSSLEQMIFSSALPTIVGELGGVEHMSWVISAFMVTMTIALPLYGKLGDGLGRKWFYISGIAFFIIGSALGGFANTMTLLIIGRAVQGFGAGAMMINSQAIIAEVVPARERGKYMGVMGAVFGISSVLGPVLGGWFTDGPGWRWGLWMNIPLGLLAMTVASIVLDLSKGNRDGFRFDWLGATFMAVSTSTLILATTWGGLQYPWGSPRIVGLLVTSAVAAALFVVVELRATDPLVPMHLFRNRNMALTTAASVVLGISMTGVMAYLPTYLQMVHSMTPTEAGLMMIPMVGGMIITSIGIGALISRTGSYKIFPIVGLGVVALGCYLLSRLTVDTGLWTLGLYIFIYGFGLGMVMQVLILIVQNSFPIAVVGTATAANNFFRQIGMSVGASVVGTVFIHNMQQNMEERLPGALAALGPEGAKYAESFSDGATQSMTPSAVNQLPQPLHDAISTSYNDGLTPIFLLLIPLVVAAALLLVPVHEDTLKETIE

SEQ ID NO: 19 - protein, 519 aa, Corynebacterium genitalium
MVETRADKQPPQATAPNVGLVFSALLLTMLMSSLGQMIFATALPTIVGELGGVDHMSWVISAFLVTMTIAMPVNGKLGDILGRKWLYITGIGLFVVGSTIGGFAHTMELLIIGRAVQGLGAGGMMVNSQSIIAEVVPARERGKYMGVMGAVFGVSSVLGPVLGGWFTDGPGWRWALWMNIPLGLLAMSVCAAVLRLRRGTAKGMHYDYLGTTLMVVATASLILTTTWGGTQYEWTSPTIIATSLIALVAAVAFVFVELRATNPLIPMDLFQNRNMVLTTLAGTVLGLAMTSGLAYLPTYLQMVHQLTPTEAGLMMLPMVIGMLVTGMTVGFIISKTGRYKIYPLVGMLITTLGLFLFSRLDVTTSLTRLGIYMFIFGFGLGLVMQVLVLIVQNSFPLKHVGTATSTNNFFRQIGSSIGASLSGSLFIHNMRDNLEQRLPEALAKLGPEGEAYAAKFQDGAANSLTPGTVAQLPDPLREAVLSSYNDGLTPVFLLMVPLTVIAFVLLLPVREEALKEDLS

SEQ ID NO: 20 - protein, 519 aa, synthetic construct
MVETRADKQPPQATAPNVGLVFSALLLTMLMSSLEQMIFATALPTIVGELGGVDHMSWVISAFLVTMTIAMPVNGKLGDILGRKWLYITGIGLFVVGSTIGGFAHTMELLIIGRAVQGLGAGGMMVNSQSIIAEVVPARERGKYMGVMGAVFGVSSVLGPVLGGWFTDGPGWRWALWMNIPLGLLAMSVCAAVLRLRRGTAKGMHYDYLGTTLMVVATASLILTTTWGGTQYEWTSPTIIATSLIALVAAVAFVFVELRATNPLIPMDLFQNRNMVLTTLAGTVLGLAMTSGLAYLPTYLQMVHQLTPTEAGLMMLPMVIGMLVTGMTVGFIISKTGRYKIYPLVGMLITTLGLFLFSRLDVTTSLTRLGIYMFIFGFGLGLVMQVLVLIVQNSFPLKHVGTATSTNNFFRQIGSSIGASLSGSLFIHNMRDNLEQRLPEALAKLGPEGEAYAAKFQDGAANSLTPGTVAQLPDPLREAVLSSYNDGLTPVFLLMVPLTVIAFVLLLPVREEALKEDLS

SEQ ID NO: 21 - protein, 549 aa, Corynebacterium glutamicum
MTSQVKPDDERPVTTISKSGAPSAHTSAPYGAAATEEAVEEKTKGRVGFIIAALMLAMLLSSLGQTIFGSALPTIVGELGGVNHMTWVITAFLLGQTISLPIFGKLGDQFGRKYLFMFAIALFVVGSIIGALAQNMTTLIVARALQGIAGGGLMILSQAITADVTTARERAKYMGIMGSVFGLSSILGPLLGGWFTDGPGWRWGLWLNVPIGIIALVAIAVLLKLPARERGKVSVDWLGSIFMAIATTAFVLAVTWGGNEYEWASPMIIGLFITTLVAAIVFVFVEKRAVDPLVPMGLFSNRNFVLTAVAGIGVGLFMMGTIAYMPTYLQMVHGLNPTQAGLMLIPMMIGLIGTSTVVGNIVSKTGKYKWYPFIGMLIMVLALVLLSTLTPSASLALIGLYFFVFGFGLGCAMQILVLIVQNSFPITMVGTATGSNNFFRQIGGAVGSALIGGLFISNLSDRFTENVPAAVASMGEEGAQYASAMSDFSGASNLTPHLVESLPQALREAIQLSYNDALTPIFLALTPIAVVAAILLFFIREDHLKETHE

SEQ ID NO: 22 - protein, 397 aa, synthetic construct
LMLAMLLSSLEQTIFGSALPTIVGELGGVNHMTWVITAFLLGQTISLPIFGKLGDQFGRKYLFMFAIALFVVGSIIGALAQNMTTLIVARALQGIAGGGLMILSQAITADVTTARERAKYMGIMGSVFGLSSILGPLLGGWFTDGPGWRWGLWLNVPIGIIALVAIAVLLKLPARERGKVSVDWLGSIFMAIATTAFVLAVTWGGNEYEWASPMIIGLFITTLVAAIVFVFVEKRAVDPLVPMGLFSNRNFVLTAVAGIGVGLFMMGTIAYMPTYLQMVHGLNPTQAGLMLIPMMIGLIGTSTVVGNIVSKTGKYKWYPFIGMLIMVLALVLLSTLTPSASLALIGLYFFVFGFGLGCAMQILVLIVQNSFPITMVGTATGSNNFFRQIGGAVGSAL

SEQ ID NO: 23 - protein, 396 aa, Corynebacterium glutamicum
LMVAMMMASLDQMIFGTALPTIVGELGGVDHMMWVITAYLLAETIMLPIYGKLGDLVGRKGLFIGALGIFLIGSVIGGLAGNMTWLIVGRAVQGIGGGGLMILSQAIIADVVPARERGRYMGVMGGVFGLSAVLGPLLGGWFTEGPGWRWAFWMNIPLGIIAIGVAIYFLDIPKKSVKFRWDYLGTFFMIVAATSLILFTTWGGSQYEWSDPIIIGLIITTIVAAALLVVVELRAKDPLVPMSFFQNRNFTLTTIAGLILGIAMFGIIGYLPTYLQMVHGINATEAGYMLIPMMVGMMGTSIWTGIRISNTGKYKLFPPIGMVVTFVALIFFARMEVSTTLWQIGIYLFVLGVGLGLAMQVLVLIVQNTLPTAVVGSATAVNNFFRQIGSSLGSAL

SEQ ID NO: 24 - protein, 396 aa, synthetic construct
LMVAMMMASLGQMIFGTALPTIVGELGGVDHMMWVITAYLLAETIMLPIYGKLGDLVGRKGLFIGALGIFLIGSVIGGLAGNMTWLIVGRAVQGIGGGGLMILSQAIIADVVPARERGRYMGVMGGVFGLSAVLGPLLGGWFTEGPGWRWAFWMNIPLGIIAIGVAIYFLDIPKKSVKFRWDYLGTFFMIVAATSLILFTTWGGSQYEWSDPIIIGLIITTIVAAALLVVVELRAKDPLVPMSFFQNRNFTLTTIAGLILGIAMFGIIGYLPTYLQMVHGINATEAGYMLIPMMVGMMGTSIWTGIRISNTGKYKLFPPIGMVVTFVALIFFARMEVSTTLWQIGIYLFVLGVGLGLAMQVLVLIVQNTLPTAVVGSATAVNNFFRQIGSSLGSAL

SEQ ID NO: 25 - protein, 397 aa, Corynebacterium pseudotuberculosis
LMVSMLLSSLDQMIFSTALPTIVGELGGVDHMMWVITAYMVGETVMLPIYGKLGDLIGRKGLFIGALIVFLIGSVFGGMAHTMTMLIAGRAIQGIGAGGLMILSQAIIADIIPARERGRYMGWMGGIFGLSAVLGPLLGGWFTEGIGWRWAFWMNLPLGAIAVAIAIYFLRIPTLEKKPFTWDYLGTVFMIIATVSLILVTTWGGSQYEWSDPLIIGLIITTIFSAGLLVLVELKATDPLIPLSFFTNRNFALTTAAGLVLGITMFGVLGYLPTYMQMVSGISATEAGYMMIPMMVGMMGLSIWSGTRIAKTGKYRHFPIIGMLVTLGALALFHTLHTSIPLWQIGLYLFTLGVGLGLSMQVLVLIVQNTLPMEVVGSATAVNNFFRQIGASLGAAL

SEQ ID NO: 26 - protein, 397 aa, synthetic construct
LMVSMLLSSLGQMIFSTALPTIVGELGGVDHMMWVITAYMVGETVMLPIYGKLGDLIGRKGLFIGALIVFLIGSVFGGMAHTMTMLIAGRAIQGIGAGGLMILSQAIIADIIPARERGRYMGWMGGIFGLSAVLGPLLGGWFTEGIGWRWAFWMNLPLGAIAVAIAIYFLRIPTLEKKPFTWDYLGTVFMIIATVSLILVTTWGGSQYEWSDPLIIGLIITTIFSAGLLVLVELKATDPLIPLSFFTNRNFALTTAAGLVLGITMFGVLGYLPTYMQMVSGISATEAGYMMIPMMVGMMGLSIWSGTRIAKTGKYRHFPIIGMLVTLGALALFHTLHTSIPLWQIGLYLFTLGVGLGLSMQVLVLIVQNTLPMEVVGSATAVNNFFRQIGASLGAAL

SEQ ID NO: 27 - protein, 396 aa, Corynebacterium kroppenstedtii
IMSAMLLASLDQMLFSTAFPTIVGDLGGVEHMSWVITSYLLCQTIMMPIYGKLGDQIGRKPIFVGAIAIFLIGSIIGGLSQSMAQLIIGRGIQGLGGGGLMILSQAIMADVVPPRERGKYAGWMGSVFGVSSVLGPVLGGWFTDGPGWRWAFWINLPVGLLAVAIALFALKLPKRGTGLKLDYFGIIFMATSASCLILFTSWGGNQYSWSSPTIIGLEIGTVVAAAIFVFIELHAKDPLIPMSLFKNRNFNLVTLGGLCVGIVMFGVMSYMPTYFQMVHNMNPTTSGFMMISMMVGLMGTSIGLGNVVTRTGKYRIYPPIGMLIVVASCVLLHRITVDTSLWYLGLCLFIMGVGLGMTMQILILVVQNSFPIQKVGVATGSNNFFRQIGSSLGSAL

SEQ ID NO: 28 - protein, 396 aa, synthetic construct
IMSAMLLASLGQMLFSTAFPTIVGDLGGVEHMSWVITSYLLCQTIMMPIYGKLGDQIGRKPIFVGAIAIFLIGSIIGGLSQSMAQLIIGRGIQGLGGGGLMILSQAIMADVVPPRERGKYAGWMGSVFGVSSVLGPVLGGWFTDGPGWRWAFWINLPVGLLAVAIALFALKLPKRGTGLKLDYFGIIFMATSASCLILFTSWGGNQYSWSSPTIIGLEIGTVVAAAIFVFIELHAKDPLIPMSLFKNRNFNLVTLGGLCVGIVMFGVMSYMPTYFQMVHNMNPTTSGFMMISMMVGLMGTSIGLGNVVTRTGKYRIYPPIGMLIVVASCVLLHRITVDTSLWYLGLCLFIMGVGLGMTMQILILVVQNSFPIQKVGVATGSNNFFRQIGSSLGSAL